European Patent Application EP 4 159 742 A1, published April 5, 2023. Title: Lactic acid bacteria growth promoter. Applicant: Asahi Group Holdings, Ltd. The sequence listing filed with the application follows.

SEQUENCE LISTING (15 sequences)

SEQ ID NO: 1 - protein, 4 aa, Saccharomyces cerevisiae
VPAF

SEQ ID NO: 2 - protein, 4 aa, Saccharomyces cerevisiae
LPWG

SEQ ID NO: 3 - protein, 9 aa, Saccharomyces cerevisiae
APKPDYPIA

SEQ ID NO: 4 - protein, 4 aa, Saccharomyces cerevisiae
PSVF

SEQ ID NO: 5 - protein, 6 aa, Saccharomyces cerevisiae
AGPQTF

SEQ ID NO: 6 - protein, 4 aa, Saccharomyces cerevisiae
IPIT

SEQ ID NO: 7 - protein, 4 aa, Saccharomyces cerevisiae
LPLG

SEQ ID NO: 8 - protein, 7 aa, Saccharomyces cerevisiae
SEYPPLG

SEQ ID NO: 9 - protein, 4 aa, Saccharomyces cerevisiae
IPGI

SEQ ID NO: 10 - protein, 4 aa, Saccharomyces cerevisiae
IPIQ

SEQ ID NO: 11 - protein, 4 aa, Saccharomyces cerevisiae
LPVL

SEQ ID NO: 12 - protein, 4 aa, Saccharomyces cerevisiae
VPVG

SEQ ID NO: 13 - protein, 7 aa, Saccharomyces cerevisiae
WDESRFQ

SEQ ID NO: 14 - protein, 9 aa, Saccharomyces cerevisiae
HDDKHIIVD

SEQ ID NO: 15 - protein, 8 aa, Saccharomyces cerevisiae
PNVLPETE